European Patent Application EP 4 799 619 A1, published September 2, 2026. Title: COMPOUND TARGETING EGR-1 AND USE THEREOF FOR TREATMENT OF ATOPIC DERMATITIS. Applicant: 주식회사 아제라메디. Application EP 24858868.3, filed March 24, 2026. The sequence listing filed with the application follows.

SEQUENCE LISTING (19 sequences)

SEQ ID NO: 1 - DNA, 27 bp, synthetic construct
  source 1..27: mol_type = other DNA
tcgcccccgctcgcccccgctggatcc

SEQ ID NO: 2 - DNA, 27 bp, synthetic construct
  source 1..27: mol_type = other DNA
ggatccagcgggggcgagcgggggcga

SEQ ID NO: 3 - DNA, 25 bp, synthetic construct
  source 1..25: mol_type = other DNA
agagtgtgtctccttcgcacacatc

SEQ ID NO: 4 - DNA, 21 bp, Homo sapiens
  source 1..21: mol_type = other DNA
tagcaatcggccacattgcct

SEQ ID NO: 5 - DNA, 21 bp, Homo sapiens
  source 1..21: mol_type = other DNA
gaagcgacgccacaatccttg

SEQ ID NO: 6 - DNA, 25 bp, Homo sapiens
  source 1..25: mol_type = other DNA
aaacagatgaagtgctccttccagg

SEQ ID NO: 7 - DNA, 24 bp, Homo sapiens
  source 1..24: mol_type = other DNA
tggagaacaccacttgttgctcca

SEQ ID NO: 8 - DNA, 20 bp, Homo sapiens
  source 1..20: mol_type = other DNA
gccttcggtccagttgcctt

SEQ ID NO: 9 - DNA, 22 bp, Homo sapiens
  source 1..22: mol_type = other DNA
agtgcctctttgctgctttcac

SEQ ID NO: 10 - DNA, 23 bp, Homo sapiens
  source 1..23: mol_type = other DNA
gacacatggatctaagagaagag

SEQ ID NO: 11 - DNA, 20 bp, Homo sapiens
  source 1..20: mol_type = other DNA
aactgactgttgtccctgag

SEQ ID NO: 12 - DNA, 24 bp, Homo sapiens
  source 1..24: mol_type = other DNA
atggcccgccgcgctgctctctcc

SEQ ID NO: 13 - DNA, 21 bp, Homo sapiens
  source 1..21: mol_type = other DNA
gttggatttgtcactgttcag

SEQ ID NO: 14 - DNA, 22 bp, Homo sapiens
  source 1..22: mol_type = other DNA
cttctgtgcctgctgctcatag

SEQ ID NO: 15 - DNA, 20 bp, Homo sapiens
  source 1..20: mol_type = other DNA
ctggacaagcaaacccaaac

SEQ ID NO: 16 - DNA, 20 bp, Homo sapiens
  source 1..20: mol_type = other DNA
acaggtaccatgaaggtctc

SEQ ID NO: 17 - DNA, 21 bp, Homo sapiens
  source 1..21: mol_type = other DNA
gcaaatttgtgtaagttcagg

SEQ ID NO: 18 - DNA, 19 bp, Homo sapiens
  source 1..19: mol_type = other DNA
acccactcctccacctttg

SEQ ID NO: 19 - DNA, 19 bp, Homo sapiens
  source 1..19: mol_type = other DNA
ctcttgtgctcttgctggg